European Patent Specification EP 3 275 891 B1, published September 3, 2025. Title: Peptide for Skin Whitening and Use Thereof. Applicant: CAREGEN CO., LTD. The sequence listing filed with the application follows.

SEQUENCE LISTING (7 sequences)

SEQ ID NO: 1 - protein, 13 aa, Apigmerin
IWSLDTQYGGRGD

SEQ ID NO: 2 - DNA, 21 bp, MITF Forward Primer
ccagcctggcgatcatgtcat

SEQ ID NO: 3 - DNA, 20 bp, MITF Reverse Primer
ggtctggacaggagttgctg

SEQ ID NO: 4 - DNA, 20 bp, Tyrosinase Forward Primer
ggccagctttcaggcagagg

SEQ ID NO: 5 - DNA, 20 bp, Tyrosinase Reverser Primer
tggtgcttcatgggcaaaat

SEQ ID NO: 6 - DNA, 20 bp, PAR2 Forward Primer
tgctagcagcctctctctcc

SEQ ID NO: 7 - DNA, 20 bp, PAR2 Reverse Primer
cttcaaggggaaccagatga